European Patent Specification EP 3 833 676 B1, published May 28, 2025. Title: POLYPEPTIDES SELF-ASSEMBLING INTO NANOPARTICLES. Applicant: ETH Zuerich. The sequence listing filed with the application follows.

SEQUENCE LISTING (38 sequences)

SEQ ID NO: 1 - protein, 186 aa, Artificial Sequence
  Synthetic sequence
  MISC_FEATURE (2)..(2): Any amino acid
  MISC_FEATURE (11)..(11): At least 3 of the X amino acids at positions 11, 39, 66, 103,, 130, and 163  are independently of each other a positively charged amino acid.
  MISC_FEATURE (28)..(28): Any amino acid
  MISC_FEATURE (30)..(30): Any amino acid
  MISC_FEATURE (39)..(39): At least 3 of the X amino acids at positions 11, 39, 66, 103,, 130, and 163  are independently of each other a positively charged amino acid.
  MISC_FEATURE (51)..(51): Any amino acid
  MISC_FEATURE (54)..(54): Any amino acid
  MISC_FEATURE (55)..(55): Any amino acid
  MISC_FEATURE (58)..(58): Any amino acid
  MISC_FEATURE (62)..(62): Any amino acid
  MISC_FEATURE (66)..(66): At least 3 of the X amino acids at positions 11, 39, 66, 103,, 130, and 163  are independently of each other a positively charged amino acid.
  MISC_FEATURE (76)..(76): Any amino acid
  MISC_FEATURE (86)..(86): Any amino acid
  MISC_FEATURE (88)..(88): Any amino acid
  MISC_FEATURE (90)..(90): Any amino acid
  MISC_FEATURE (92)..(92): Any amino acid
  MISC_FEATURE (93)..(93): Any amino acid
  MISC_FEATURE (94)..(94): Any amino acid
  MISC_FEATURE (103)..(103): At least 3 of the X amino acids at positions 11, 39, 66, 103,, 130, and 163  are independently of each other a positively charged amino acid.
  MISC_FEATURE (114)..(114): Any amino acid
  MISC_FEATURE (117)..(117): Any amino acid
  MISC_FEATURE (120)..(120): Any amino acid
  MISC_FEATURE (130)..(130): At least 3 of the X amino acids at positions 11, 39, 66, 103,, 130, and 163  are independently of each other a positively charged amino acid.
  MISC_FEATURE (163)..(163): At least 3 of the X amino acids at positions 11, 39, 66, 103,, 130, and 163  are independently of each other a positively charged amino acid.
  MISC_FEATURE (172)..(172): Any amino acid
  MISC_FEATURE (175)..(175): Any amino acid
  MISC_FEATURE (179)..(179): Any amino acid
  MISC_FEATURE (183)..(183): Any amino acid
  MISC_FEATURE (185)..(185): Any amino acid
MXQAIGILELXSIAAGMELGDAMLKSAXVXLLVSKTISXGKFLLMLGGDIXAIXXAIXTGTXQAGXLLVDSLVLAXIHPSVLPAIXGXNXVXXXQAVGIVETXSVAACISAADXAVXGSXVTLVRVHMAXGIGGKCYMVVAGDVSDVALAVTVASSSAGAYGXLVYASLIPXPHXAMWXQMVXGXE

SEQ ID NO: 2 - protein, 192 aa, Artificial Sequence
  Synthetic sequence
MSQAIGILELRSIAAGMELGDAMLKSANVDLLVSKTISRGKFLLMLGGDIGAIQQAIETGTSQAGRLLVDSLVLANIHPSVLPAISGLNSVDKRQAVGIVETRSVAACISAADRAVKGSNVTLVRVHMARGIGGKCYMVVAGDVSDVALAVTVASSSAGAYGRLVYASLIPRPHEAMWRQMVEGLEHHHHHH

SEQ ID NO: 3 - protein, 188 aa, Artificial Sequence
  Synthetic sequence
MSQAIGILELRSIAAGMELGDAMLKSANVDLLVSKTISRGKFLLMLGGDIGAIQQAIETGTSQAGRLLVDSLVLANIHPSVLPAISGLNSVDKRQAVGIVETRSVAACISAADRAVKGSNVTLVRVHMARGIGGKCYMVVAGDVSDVALAVTVASSSAGAYGRLVYASLIPRPHEAMWRQMVEGLEGS

SEQ ID NO: 4 - protein, 192 aa, Artificial Sequence
  Synthetic sequence
MSQAIGILELRSIAAGMELGDAMLKSANVDLLVSKTISRGKFLLMLGGDIGAIQQAIETGTSQAGRLLVDSLVLANIHPSVLPAISGLNSVDCRQAVGIVETRSVAACISAADRAVKGSNVTLVRVHMARGIGGKCYMVVAGDVSDVALAVTVASSSAGAYGRLVYASLIPRPHEAMWRQMVEGLEHHHHHH

SEQ ID NO: 5 - protein, 230 aa, Artificial Sequence
  Synthetic sequence
MSQAIGILELRSIAAGMELGDAMLKSANVDLLVSKTISRGKFLLMLGGDIGAIQQAIETGTSQAGRLLVDSLVLANIHPSVLPAISGLNSVDCRQAVGIVETRSVAACISAADRAVKGSNVTLVRVHMARGIGGKCYMVVAGDVSDVALAVTVASSSAGAYGRLVYASLIPRPHEAMWRQMVEGLEHHHHHHEFPPEVEEQDDGTLPMSCAQESGMDRHPAACASARINV

SEQ ID NO: 6 - protein, 192 aa, Artificial Sequence
  Synthetic sequence
MSQAIGILELTSIAAGMELGDAMLKSANVDLLVSKTISRGKFLLMLGGDIGAIQQAIETGTSQAGELLVDSLVLANIHPSVLPAISGLNSVDKRQAVGIVETWSVAACISAADRAVKGSNVTLVRVHMAFGIGGKCYMVVAGDVSDVALAVTVASSSAGAYGLLVYASLIPRPHEAMWRQMVEGLEHHHHHH

SEQ ID NO: 7 - protein, 192 aa, Artificial Sequence
  Synthetic sequence
MSQAIGILELTSIAAGMELGDAMLKSANVDLLVSKTISRGKFLLMLGGDIGAIQQAIETGTSQAGELLVDSLVLANIHPSVLPAISGLNSVDKRQAVGIVETWSVAACISAADRAVKGSNVTLVRVHMARGIGGKCYMVVAGDVSDVALAVTVASSSAGAYGLLVYASLIPRPHEAMWRQMVEGLEHHHHHH

SEQ ID NO: 8 - protein, 192 aa, Artificial Sequence
  Synthetic sequence
MSQAIGILELRSIAAGMELGDAMLKSANVDLLVSKTISPGKFLLMLGGDIGAIQQAIETGTSQAGELLVDSLVLANIHPSVLPAISGLNSVDKRQAVGIVETRSVAACISAADRAVKGSNVTLVRVHMAFGIGGKCYMVVAGDVSDVALAVTVASSSAGAYGLLVYASLIPRPHEAMWRQMVEGLEHHHHHH

SEQ ID NO: 9 - protein, 192 aa, Artificial Sequence
  Synthetic sequence
MSQAIGILELRSIAAGMELGDAMLKSANVDLLVSKTISRGKFLLMLGGDIGAIQQAIETGTSQAGELLVDSLVLANIHPSVLPAISGLNSVDKRQAVGIVETWSVAACISAADRAVKGSNVTLVRVHMAFGIGGKCYMVVAGDVSDVALAVTVASSSAGAYGLLVYASLIPRPHEAMWRQMVEGLEHHHHHH

SEQ ID NO: 10 - protein, 192 aa, Artificial Sequence
  Synthetic sequence
MSQAIGILELTSIAAGMELGDAMLKSANVDLLVSKTISPGKFLLMLGGDIGAIQQAIETGTSQAGELLVDSLVLANIHPSVLPAISGLNSVDKRQAVGIVETRSVAACISAADRAVKGSNVTLVRVHMARGIGGKCYMVVAGDVSDVALAVTVASSSAGAYGRLVYASLIPRPHEAMWRQMVEGLEHHHHHH

SEQ ID NO: 11 - protein, 191 aa, Artificial Sequence
  Synthetic sequence
MSQAIGILELRSIAAGMELGDAMLKSANVDLLVSKTISRGKFLLMLGGDIGAIQQAIETGTSQAGELLVDSLVLANIHPSVLPAISGLNSVDKRQAVGIVETWSVAACISAADRAVKGSNVTLVRVHMARGIGGKCYMVVAGDVSDVALAVTVASSSAGAYGLLVYASLIPRPHEAMWRQMVEGLEHHHHH

SEQ ID NO: 12 - protein, 192 aa, Artificial Sequence
  Synthetic sequence
MSQAIGILELRSIAAGMELGDAMLKSANVDLLVSKTISRGKFLLMLGGDIGAIQQAIETGTSQAGELLVDSLVLANIHPSVLPAISGLNSVDKRQAVGIVETRSVAACISAADRAVKGSNVTLVRVHMARGIGGKCYMVVAGDVSDVALAVTVASSSAGAYGLLVYASLIPRPHEAMWRQMVEGLEHHHHHH

SEQ ID NO: 13 - protein, 192 aa, Artificial Sequence
  Synthetic sequence
MSQAIGILELRSIAAGMELGDAMLKSANVDLLVSKTISPGKFLLMLGGDIGAIQQAIETGTSQAGRLLVDSLVLANIHPSVLPAISGLNSVDKRQAVGIVETRSVAACISAADRAVKGSNVTLVRVHMAFGIGGKCYMVVAGDVSDVALAVTVASSSAGAYGRLVYASLIPRPHEAMWRQMVEGLEHHHHHH

SEQ ID NO: 14 - protein, 192 aa, Artificial Sequence
  Synthetic sequence
MSQAIGILELRSIAAGMELGDAMLKSANVDLLVSKTISPGKFLLMLGGDIGAIQQAIETGTSQAGRLLVDSLVLANIHPSVLPAISGLNSVDKRQAVGIVETRSVAACISAADRAVKGSNVTLVRVHMARGIGGKCYMVVAGDVSDVALAVTVASSSAGAYGRLVYASLIPRPHEAMWRQMVEGLEHHHHHH

SEQ ID NO: 15 - protein, 192 aa, Artificial Sequence
  Synthetic sequence
MSQAIGILELRSIAAGMELGDAMLKSANVDLLVSKTISRGKFLLMLGGDIGAIQQAIETGTSQAGRLLVDSLVLANIHPSVLPAISGLNSVDKRQAVGIVETWSVAACISAADRAVKGSNVTLVRVHMARGIGGKCYMVVAGDVSDVALAVTVASSSAGAYGRLVYASLIPRPHEAMWRQMVEGLEHHHHHH

SEQ ID NO: 16 - protein, 192 aa, Artificial Sequence
  Synthetic sequence
MSQAIGILELRSIAAGMELGDAMLKSANVDLLVSKTISRGKFLLMLGGDIGAIQQAIETGTSQAGRLLVDSLVLANIHPSVLPAISGLNSVDKRQAVGIVETRSVAACISAADRAVKGSNVTLVRVHMARGIGGKCYMVVAGDVSDVALAVTVASSSAGAYGLLVYASLIPRPHEAMWRQMVEGLEHHHHHH

SEQ ID NO: 17 - protein, 38 aa, Artificial Sequence
  Synthetic sequence
EFPPEVEEQDDGTLPMSCAQESGMDRHPAACASARINV

SEQ ID NO: 18 - DNA, 21 bp, Artificial Sequence
  Synthetic sequence
ttaattaaagacttcaagcgg

SEQ ID NO: 19 - DNA, 21 bp, Artificial Sequence
  Synthetic sequence
gcttgaagtctttaattaatt

SEQ ID NO: 20 - DNA, 21 bp, Artificial Sequence
  Synthetic sequence
gaacttcagggtcagcttggg

SEQ ID NO: 21 - DNA, 21 bp, Artificial Sequence
  Synthetic sequence
caagctgaccctgaagttctt

SEQ ID NO: 22 - DNA, 21 bp, Artificial Sequence
  Synthetic sequence
gaacttcagggtcagcttggg

SEQ ID NO: 23 - DNA, 21 bp, Artificial Sequence
  Synthetic sequence
caagctgaccctgaagttctt

SEQ ID NO: 24 - DNA, 21 bp, Artificial Sequence
  Synthetic sequence
uaaggcuaugaagagauactt

SEQ ID NO: 25 - DNA, 20 bp, Artificial Sequence
  Synthetic sequence
guaucuuucauagccuuatt

SEQ ID NO: 26 - DNA, 18 bp, Artificial Sequence
  Synthetic sequence
tcgagggcagctaatgag

SEQ ID NO: 27 - DNA, 18 bp, Artificial Sequence
  Synthetic sequence
tgcactcattagctgccc

SEQ ID NO: 28 - DNA, 18 bp, Artificial Sequence
  Synthetic sequence
cgtggcgagcagcagcgc

SEQ ID NO: 29 - DNA, 20 bp, Artificial Sequence
  Synthetic sequence
cctggtgcgtgtgcacatgg

SEQ ID NO: 30 - DNA, 22 bp, Artificial Sequence
  Synthetic sequence
gtgctcgagaccttccaccatc

SEQ ID NO: 31 - DNA, 23 bp, Artificial Sequence
  Synthetic sequence
ggtgatgcgatgctgaaaagcgc

SEQ ID NO: 32 - DNA, 24 bp, Artificial Sequence
  Synthetic sequence
gcgattcagcaggcgattgaaacc

SEQ ID NO: 33 - DNA, 24 bp, Artificial Sequence
  Synthetic sequence
cgattagcggtctgaatagcgtgg

SEQ ID NO: 34 - DNA, 24 bp, Artificial Sequence
  Synthetic sequence
ggtttcaatcgcctgctgaatcgc

SEQ ID NO: 35 - DNA, 24 bp, Artificial Sequence
  Synthetic sequence
ccacgctattcagaccgctaatcg

SEQ ID NO: 36 - DNA, 26 bp, Artificial Sequence
  Synthetic sequence
gaaggagatatacatatgagccaggc

SEQ ID NO: 37 - protein, 189 aa, Artificial Sequence
  Synthetic sequence
MSQAIGILELRSIAAGMELGDAMLKSANVDLLVSKTISRGKFLLMLGGDIGAIQQAIETGTSQAGRLLVDSLVLANIHPSVLPAISGLNSVDKRQAVGIVETRSVAACISAADRAVKGSNVTLVRVHMARGIGGKCYMVVAGDVSDVALAVTVASSSAGAYGRLVYASLIPRPHEAMWRQMVEGLEHHH

SEQ ID NO: 38 - protein, 195 aa, Artificial Sequence
  Synthetic sequence
MSQAIGILELRSIAAGMELGDAMLKSANVDLLVSKTISRGKFLLMLGGDIGAIQQAIETGTSQAGRLLVDSLVLANIHPSVLPAISGLNSVDKRQAVGIVETRSVAACISAADRAVKGSNVTLVRVHMARGIGGKCYMVVAGDVSDVALAVTVASSSAGAYGRLVYASLIPRPHEAMWRQMVEGLEHHHHHHHHH